European Patent Application EP 4 148 135 A1, published March 15, 2023. Title: U1 SNRNP REGULATES GENE EXPRESSION AND MODULATES ONCOGENICITY. Applicant: The Trustees of the University of Pennsylvania. The sequence listing filed with the application follows.

SEQUENCE LISTING (63 sequences)

SEQ ID NO: 1 - DNA, 9 bp, Artificial Sequence
  Wild-type 5' splice site recognition sequence of U1
acttacctg

SEQ ID NO: 2 - DNA, 9 bp, Artificial Sequence
  U1-A: mutated 5' splice site recognition sequence of U1
ctgctgttg

SEQ ID NO: 3 - DNA, 9 bp, Artificial Sequence
  U1-B: mutated 5' splice site recognition sequence of U1
tgaatggac

SEQ ID NO: 4 - DNA, 9 bp, Artificial Sequence
  U1-C: mutated 5' splice site recognition sequence of U1
ctacagatg

SEQ ID NO: 5 - DNA, 9 bp, Artificial Sequence
  U1-D: mutated 5' splice site recognition sequence of U1
cacccctac

SEQ ID NO: 6 - DNA, 25 bp, Artificial Sequence
  Chemically synthesized
cctcttacctcagttacaatttata

SEQ ID NO: 7 - DNA, 25 bp, Artificial Sequence
  Chemically synthesized
ggtatctcccctgccaggtaagtat

SEQ ID NO: 8 - DNA, 25 bp, Artificial Sequence
  Chemically synthesized
tgataagaacagatactacacttga

SEQ ID NO: 9 - DNA, 25 bp, Artificial Sequence
  Chemically synthesized
aaccttctctcctttcatacaacac

SEQ ID NO: 10 - DNA, 24 bp, Artificial Sequence
  Chemically synthesized
tcgttattttccttactcataagt

SEQ ID NO: 11 - DNA, 25 bp, Artificial Sequence
  Chemically synthesized
gttaacctctacgccaggtaagtat

SEQ ID NO: 12 - DNA, 25 bp, Artificial Sequence
  Chemically synthesized
gataagaacagatactacactttga

SEQ ID NO: 13 - DNA, 25 bp, Artificial Sequence
  Chemically synthesized
aacttgctctccttccaaacaacac

SEQ ID NO: 14 - DNA, 25 bp, Artificial Sequence
  Chemically synthesized
gattggttttccttactcattagtt

SEQ ID NO: 15 - DNA, 25 bp, Artificial Sequence
  Chemically synthesized
ggatattttcttcctaaaaggaatc

SEQ ID NO: 16 - DNA, 25 bp, Artificial Sequence
  Chemically synthesized
aataccacagtttattgaagactac

SEQ ID NO: 17 - DNA, 59 bp, Artificial Sequence
  Chemically synthesized
cgtatcgcctccctcgcgccatcagacgagtgcgtgctcgagcggccgcccgggcaggt

SEQ ID NO: 18 - DNA, 58 bp, Artificial Sequence
  Chemically synthesized
ctatgcgccttgccagcccgctcagacgagtgcgtggcagcgtggtcgcggccgaggt

SEQ ID NO: 19 - DNA, 59 bp, Artificial Sequence
  Chemically synthesized
cgtatcgcctccctcgcgccatcagacgctcgacagctcgagcggccgcccgggcaggt

SEQ ID NO: 20 - DNA, 58 bp, Artificial Sequence
  Chemically synthesized
ctatgcgccttgccagcccgctcagacgctcgacaggcagcgtggtcgcggccgaggt

SEQ ID NO: 21 - DNA, 20 bp, Artificial Sequence
  Chemically synthesized
cagtctgccattgtgacgtg

SEQ ID NO: 22 - DNA, 20 bp, Artificial Sequence
  Chemically synthesized
ccaatgggagagccctaaac

SEQ ID NO: 23 - DNA, 19 bp, Artificial Sequence
  Chemically synthesized
ctgcaatgggagttgggag

SEQ ID NO: 24 - DNA, 21 bp, Artificial Sequence
  Chemically synthesized
gatgcgtttgattctgcccac

SEQ ID NO: 25 - DNA, 25 bp, Artificial Sequence
  Chemically synthesized
gaggagctctccaaactgatcagcg

SEQ ID NO: 26 - DNA, 20 bp, Artificial Sequence
  Chemically synthesized
ctgatcagcggctttgacca

SEQ ID NO: 27 - DNA, 27 bp, Artificial Sequence
  Chemically synthesized
cgagtatgagtcgactctagactgccg

SEQ ID NO: 28 - DNA, 21 bp, Artificial Sequence
  Chemically synthesized
ctctagactgccgcgacgtgg

SEQ ID NO: 29 - DNA, 40 bp, Artificial Sequence
  Chemically synthesized
ctgatctagaggtaccggatcctttttttttttttttttt

SEQ ID NO: 30 - DNA, 22 bp, Artificial Sequence
  Chemically synthesized
ctgatctagaggtaccggatcc

SEQ ID NO: 31 - DNA, 25 bp, Artificial Sequence
  Chemically synthesized
gctaactcaggggctgcataggcac

SEQ ID NO: 32 - DNA, 25 bp, Artificial Sequence
  Chemically synthesized
cgtccttctcgccctccttctcctc

SEQ ID NO: 33 - DNA, 23 bp, Artificial Sequence
  Chemically synthesized
gggtggctttcttaatttgcatc

SEQ ID NO: 34 - DNA, 22 bp, Artificial Sequence
  Chemically synthesized
gatgatttccattgctgccacg

SEQ ID NO: 35 - DNA, 25 bp, Artificial Sequence
  Chemically synthesized
gtcttgaaaccacagcagtgcccag

SEQ ID NO: 36 - DNA, 25 bp, Artificial Sequence
  Chemically synthesized
ctcagcactgacggccttgttgagt

SEQ ID NO: 37 - DNA, 24 bp, Artificial Sequence
  Chemically synthesized
cagacgatgagagaacacccgatg

SEQ ID NO: 38 - DNA, 23 bp, Artificial Sequence
  Chemically synthesized
tggcacctctgtgggcctgtggc

SEQ ID NO: 39 - DNA, 27 bp, Artificial Sequence
  Chemically synthesized
ctgttgcttccactgcttcacattggc

SEQ ID NO: 40 - DNA, 22 bp, Artificial Sequence
  Chemically synthesized
aaggataagcagtgtgaacaag

SEQ ID NO: 41 - DNA, 20 bp, Artificial Sequence
  Chemically synthesized
tctagatctcccatcacggc

SEQ ID NO: 42 - DNA, 20 bp, Artificial Sequence
  Chemically synthesized
cagcagtgccgaaagacata

SEQ ID NO: 43 - DNA, 26 bp, Artificial Sequence
  Chemically synthesized
cgcctatcagtctgtccctggactcc

SEQ ID NO: 44 - DNA, 25 bp, Artificial Sequence
  Chemically synthesized
ccttcctttggtaaggaggctgccc

SEQ ID NO: 45 - DNA, 22 bp, Artificial Sequence
  Chemically synthesized
ccggaattgctgagtaagctgg

SEQ ID NO: 46 - DNA, 23 bp, Artificial Sequence
  Chemically synthesized
ggaaggcatatactggcaaatgc

SEQ ID NO: 47 - DNA, 24 bp, Artificial Sequence
  Chemically synthesized
cctttagctcctcgaatttaacag

SEQ ID NO: 48 - DNA, 24 bp, Artificial Sequence
  Chemically synthesized
ccttgatgaacttcctcagaggac

SEQ ID NO: 49 - DNA, 21 bp, Artificial Sequence
  Chemically synthesized
ggttggtgatggtggtactgg

SEQ ID NO: 50 - DNA, 23 bp, Artificial Sequence
  Chemically synthesized
gatttcgccttcactttcctgtc

SEQ ID NO: 51 - DNA, 29 bp, Artificial Sequence
  Chemically synthesized
gtgtggatgtagtacacatggatgaaaac

SEQ ID NO: 52 - DNA, 28 bp, Artificial Sequence
  Chemically synthesized
ttattgtacaccaggaccttctccacag

SEQ ID NO: 53 - DNA, 28 bp, Artificial Sequence
  Chemically synthesized
caactatggctgtggagaaggtcctggt

SEQ ID NO: 54 - DNA, 31 bp, Artificial Sequence
  Chemically synthesized
tctgacctggagacgaaactgtagagtatct

SEQ ID NO: 55 - DNA, 22 bp, Artificial Sequence
  Chemically synthesized
caacagacattgctgaagaaac

SEQ ID NO: 56 - DNA, 18 bp, Artificial Sequence
  Chemically synthesized
attttggatgactgcggc

SEQ ID NO: 57 - DNA, 21 bp, Artificial Sequence
  Chemically synthesized
ctttaggagctgctgtcgata

SEQ ID NO: 58 - DNA, 21 bp, Artificial Sequence
  Chemically synthesized
gctcctacctcttccaagcag

SEQ ID NO: 59 - DNA, 19 bp, Artificial Sequence
  Chemically synthesized
acaaaacacagcccccagc

SEQ ID NO: 60 - DNA, 24 bp, Artificial Sequence
  Chemically synthesized
tggtgtgaatgtcagtgtgaatgc

SEQ ID NO: 61 - DNA, 22 bp, Artificial Sequence
  Chemically synthesized
gcaagttgaaggaagcagcagg

SEQ ID NO: 62 - DNA, 21 bp, Artificial Sequence
  Chemically synthesized
tgatcacgaaggtggttttcc

SEQ ID NO: 63 - DNA, 19 bp, Artificial Sequence
  Chemically synthesized
gcacatccggagtgcaatg